European Patent Specification EP 3 472 325 B1, published April 3, 2024. Title: Method for targeted DNA alteration in plant cells. Applicant: Keygene N.V. The sequence listing filed with the application follows.

SEQUENCE LISTING (8 sequences)

SEQ ID NO: 1 - DNA, 20 bp, Artificial Sequence
  sgRNA
ttactgcattccatactcga

SEQ ID NO: 2 - protein, 1435 aa, Artificial Sequence
  CAS9
MGWTLNSAGYLLGKINLKALAALAKKILAMGSSHHHHHHVYPYDVPDYAELPPKKKRKVGIENLYFQGDKKYSIGLDIGTNSVGWAVITDEYKVPSKKFKVLGNTDRHSIKKNLIGALLFDSGETAEATRLKRTARRRYTRRKNRICYLQEIFSNEMAKVDDSFFHRLEESFLVEEDKKHERHPIFGNIVDEVAYHEKYPTIYHLRKKLVDSTDKADLRLIYLALAHMIKFRGHFLIEGDLNPDNSDVDKLFIQLVQTYNQLFEENPINASGVDAKAILSARLSKSRRLENLIAQLPGEKKNGLFGNLIALSLGLTPNFKSNFDLAEDAKLQLSKDTYDDDLDNLLAQIGDQYADLFLAAKNLSDAILLSDILRVNTEITKAPLSASMIKRYDEHHQDLTLLKALVRQQLPEKYKEIFFDQSKNGYAGYIDGGASQEEFYKFIKPILEKMDGTEELLVKLNREDLLRKQRTFDNGSIPHQIHLGELHAILRRQEDFYPFLKDNREKIEKILTFRIPYYVGPLARGNSRFAWMTRKSEETITPWNFEEVVDKGASAQSFIERMTNFDKNLPNEKVLPKHSLLYEYFTVYNELTKVKYVTEGMRKPAFLSGEQKKAIVDLLFKTNRKVTVKQLKEDYFKKIECFDSVEISGVEDRFNASLGTYHDLLKIIKDKDFLDNEENEDILEDIVLTLTLFEDREMIEERLKTYAHLFDDKVMKQLKRRRYTGWGRLSRKLINGIRDKQSGKTILDFLKSDGFANRNFMQLIHDDSLTFKEDIQKAQVSGQGDSLHEHIANLAGSPAIKKGILQTVKVVDELVKVMGRHKPENIVIEMARENQTTQKGQKNSRERMKRIEEGIKELGSQILKEHPVENTQLQNEKLYLYYLQNGRDMYVDQELDINRLSDYDVDHIVPQSFLKDDSIDNKVLTRSDKNRGKSDNVPSEEVVKKMKNYWRQLLNAKLITQRKFDNLTKAERGGLSELDKAGFIKRQLVETRQITKHVAQILDSRMNTKYDENDKLIREVKVITLKSKLVSDFRKDFQFYKVREINNYHHAHDAYLNAVVGTALIKKYPKLESEFVYGDYKVYDVRKMIAKSEQEIGKATAKYFFYSNIMNFFKTEITLANGEIRKRPLIETNGETGEIVWDKGRDFATVRKVLSMPQVNIVKKTEVQTGGFSKESILPKRNSDKLIARKKDWDPKKYGGFDSPTVAYSVLVVAKVEKGKSKKLKSVKELLGITIMERSSFEKNPIDFLEAKGYKEVKKDLIIKLPKYSLFELENGRKRMLASAGELQKGNELALPSKYVNFLYLASHYEKLKGSPEDNEQKQLFVEQHKHYLDEIIEQISEFSKRVILADANLDKVLSAYNKHRDKPIREQAENIIHLFTLTNLGAPAAFKYFDTTIDRKRYTSTKEVLDATLIHQSITGLYETRIDLSQLGGD

SEQ ID NO: 3 - DNA, 4173 bp, Artificial Sequence
  op
atgggaagaggatcgcatcaccaccatcatcataagcttccaaagaagaagaggaaggttctcgagatggataagaagtactctatcggacttgatatcggaactaactctgtgggatgggctgtgatcactgatgagtacaaggtgccatctaagaagttcaaggttttgggaaacactgataggcactctatcaagaaaaaccttatcggagctttgcttttcgattctggtgagactgctgaggctactaggcttaagaggactgctagaagaaggtacactagaagaaagaacaggatctgctaccttcaagagatcttctctaacgagatggctaaagtggatgattcattcttccacaggcttgaagagtctttcttggtggaagaagataagaagcacgagaggcacccaatcttcggaaacatcgttgatgaggtggcataccacgagaagtacccaactatctaccaccttaggaagaagcttgttgattctactgataaggctgatcttaggcttatctaccttgctcttgctcacatgatcaagttcaggggacacttccttatcgagggtgatcttaacccagataactctgatgtggataagcttttcatccagcttgtgcagacttacaaccagcttttcgaagagaacccaatcaacgcttctggtgtggatgctaaggctatcctttctgctaggctttctaagtctagaaggcttgagaaccttattgctcagcttccaggtgagaagaagaacggacttttcggaaacttgatcgctctttctcttggacttactccaaacttcaagtctaacttcgatcttgctgaggatgcaaagcttcagttgtctaaggatacttacgatgatgatcttgataacttgcttgctcagatcggagatcagtacgctgatcttttccttgctgctaaaaacctttctgatgctatcttgctttctgatatccttagggtgaacactgagatcactaaggctccactttctgcttctatgatcaagaggtacgatgagcaccaccaggatcttactttgcttaaggctcttgtgaggcagcagttgccagagaagtacaaagagattttcttcgatcagtctaagaacggatacgctggttacatcgatggtggtgcatctcaagaagagttctacaagttcatcaagccaatccttgagaagatggatggaactgaagagttgcttgtgaagcttaacagagaggatcttcttaggaagcagaggactttcgataacggatctatccctcaccagatccaccttggagagcttcacgctatcttgagaaggcaagaggatttctacccattcttgaaggataacagggaaaaaatcgagaagattcttactttcaggatcccttactacgtgggaccacttgctaggggaaattctaggttcgcttggatgactaggaagtctgaagagactatcactccatggaacttcgaagaggtggtggataagggtgctagtgctcagtctttcatcgagaggatgacaaacttcgataagaaccttccaaacgagaaggtgttgccaaagcactctttgctttacgagtacttcactgtgtacaacgagcttactaaggtgaagtacgtgacagagggaatgaggaagccagctttcttgtctggtgagcaaaagaaggctatcgttgatcttttgttcaagactaatagaaaggtgacagtgaagcagcttaaagaggattacttcaaaaagatcgagtgcttcgattcagttgagatctctggtgttgaggataggttcaacgcatctttgggaacttaccacgatttgttgaagattatcaaggataaggatttcttggataacgaggaaaacgaggatatcttggaggatatcgtgcttactcttactcttttcgaggatagagagatgattgaagaaaggcttaaaacttacgctcaccttttcgatgataaggtgatgaagcagttgaagagaagaagatacacaggttggggaaggttgtctaggaagcttatcaacggaatcagggataagcagtctggtaagactatcttggatttccttaagtctgatggattcgctaataggaacttcatgcagttgatccacgatgattctttgactttcaaagaggatatccagaaggctcaggtttcaggacagggtgatagtttacacgagcacattgctaaccttgctggatctcctgcaatcaagaagggaatcttgcagactgtgaaggttgtggatgagttggtgaaggtgatgggaaggcataagccagagaacatcgtgatcgaaatggctagagagaaccagactactcagaagggacagaagaactctagggaaaggatgaagaggatcgaagagggaatcaaagagcttggatctcagatccttaaagagcacccagttgagaacactcagcttcagaacgagaagctttacctttactacttgcagaacggaagggatatgtatgtggatcaagagttggatatcaacaggttgtctgattatgatgttgatcacatcgtgccacagtcttttttgaaggatgattctatcgataacaaggtgttgactaggtctgataagaacaggggaaagtctgataacgttccatctgaagaggttgtgaaaaagatgaagaactattggaggcagcttcttaacgctaagttgatcactcagaggaagttcgataatttgactaaggctgagaggggaggattgtctgagcttgataaggcaggattcatcaagaggcagttggttgagactaggcagatcacaaagcacgtggcacagatccttgattctaggatgaacactaagtatgatgagaacgataagttaatcagggaagttaaggtgatcactttgaagtctaagcttgtgtctgattttaggaaggatttccaattctacaaggtgagagagatcaacaactaccaccacgctcacgatgcttaccttaacgctgttgtgggaactgctttgatcaagaagtatccaaagttggagtctgagttcgtgtacggtgattacaaggtgtacgatgtgaggaagatgatcgctaagtcagagcaagagatcggaaaggctactgctaagtatttcttctactctaacatcatgaatttcttcaagacagagatcactcttgctaacggtgagattaggaagaggccacttatcgagacaaatggtgagacaggtgagatcgtgtgggataagggaagggatttcgctactgtgagaaaggtgttgtctatgccacaggtgaacattgtgaagaaaactgaggtgcagactggtggattctctaaagagtctatccttccaaagaggaactctgataagttgattgctaggaaaaaggattgggatccaaaaaagtacggtggattcgattctccaactgtggcttactctgtgcttgtggtggctaaggttgagaagggaaaatcaaagaaattgaagtctgtgaaagagcttcttggaatcactatcatggaaaggtcatctttcgagaagaaccctatcgatttccttgaggctaagggatacaaagaggtgaagaaggatcttatcatcaagcttccaaagtactcacttttcgagcttgagaatggaagaaagaggatgcttgcttctgctggtgagttgcagaagggtaacgaacttgctttgccttctaagtacgttaacttcctttaccttgcttctcactacgagaagttgaagggatctccagaggataacgaacaaaagcagttgttcgttgagcagcacaagcactaccttgatgagatcatcgagcagatctctgagttctctaagagggttatcttggctgatgcaaaccttgataaggtgttgagtgcttacaacaaacatagggataagccaatcagagagcaggctgagaacatcatccaccttttcactttgactaaccttggtgctccagctgctttcaagtacttcgatacaactattgatagaaagaggtacacttctacaaaagaggttttggatgctactttgatccaccagagtatcactggactttacgagactaggatcgatttgtctcagcttggtggtgattga

SEQ ID NO: 4 - DNA, 221 bp, Artificial Sequence
  total
ggagtgatcaaaagtcccacatcgatcaggtgatatatagcagcttagtttatataatgatagagtcgacatagcgattgttactgcattccatactcgagttttagagctagaaatagcaagttaaaataaggctagtccgttatcaacttgaaaaagtggcaccgagtcggtgctttttttctagacccagctttcttgtacaaagttggcattacgct

SEQ ID NO: 5 - DNA, 44 bp, Artificial Sequence
  p
ggatcctaatacgactcactatagttactgcattccatactcga

SEQ ID NO: 6 - DNA, 19 bp, Artificial Sequence
  .
aaaaaaagcaccgactcgg

SEQ ID NO: 7 - DNA, 21 bp, Artificial Sequence
  .
aaggtgaagggggtaaaatgg

SEQ ID NO: 8 - DNA, 22 bp, Artificial Sequence
  .
gaaggtgaagggggtaaaatgg